European Patent Specification EP 3 774 848 B1, published February 22, 2023. Title: Cyclic peptides and uses thereof. Applicant: Lateral IP Pty Ltd. The sequence listing filed with the application follows.

SEQUENCE LISTING (35 sequences)

SEQ ID NO: 1 - protein, 12 aa, Synthetic
  X (1)..(1): selected from the group consisting of serine and SEQ ID NOs:2-11
  X (4)..(4): serine, alanine, valine, leucine, isoleucine or glycine
  X (5)..(5): alanine, arginine or lysine
  X (7)..(7): serine, alanine, valine, leucine, isoleucine or glycine
  X (8)..(8): glutamic acid or aspartic acid
  X (9)..(9): serine, alanine, valine, leucine, isoleucine or glycine
  X (10)..(10): serine, alanine, valine, leucine, isoleucine or glycine
  X (12)..(12): selected from the group consisting on serine and SEQ ID NOs:12-25
XCRXXPXXXXCX

SEQ ID NO: 2 - protein, 2 aa, Synthetic
HS

SEQ ID NO: 3 - protein, 3 aa, Synthetic
GHS

SEQ ID NO: 4 - protein, 4 aa, Synthetic
PGHS

SEQ ID NO: 5 - protein, 5 aa, Synthetic
APGHS

SEQ ID NO: 6 - protein, 6 aa, Synthetic
EAPGHS

SEQ ID NO: 7 - protein, 7 aa, Synthetic
SEAPGHS

SEQ ID NO: 8 - protein, 8 aa, Synthetic
SSEAPGHS

SEQ ID NO: 9 - protein, 9 aa, Synthetic
PSSEAPGHS

SEQ ID NO: 10 - protein, 10 aa, Synthetic
DPSSEAPGHS

SEQ ID NO: 11 - protein, 11 aa, Synthetic
IDPSSEAPGHS

SEQ ID NO: 12 - protein, 2 aa, Synthetic
SS

SEQ ID NO: 13 - protein, 3 aa, Synthetic
SSK

SEQ ID NO: 14 - protein, 4 aa, Synthetic
SSKF

SEQ ID NO: 15 - protein, 5 aa, Synthetic
SSKFS

SEQ ID NO: 16 - protein, 6 aa, Synthetic
SSKFSW

SEQ ID NO: 17 - protein, 7 aa, Synthetic
SSKFSWD

SEQ ID NO: 18 - protein, 8 aa, Synthetic
SSKFSWDE

SEQ ID NO: 19 - protein, 9 aa, Synthetic
SSKFSWDEY

SEQ ID NO: 20 - protein, 10 aa, Synthetic
SSKFSWDEYE

SEQ ID NO: 21 - protein, 11 aa, Synthetic
SSKFSWDEYEQ

SEQ ID NO: 22 - protein, 12 aa, Synthetic
SSKFSWDEYEQY

SEQ ID NO: 23 - protein, 13 aa, Synthetic
SSKFSWDEYEQYK

SEQ ID NO: 24 - protein, 14 aa, Synthetic
SSKFSWDEYEQYKK

SEQ ID NO: 25 - protein, 15 aa, Synthetic
SSKFSWDEYEQYKKE

SEQ ID NO: 26 - protein, 11 aa, Synthetic
SCRSRPVESSC

SEQ ID NO: 27 - protein, 10 aa, Synthetic
CRSRPVESSC

SEQ ID NO: 28 - protein, 11 aa, Synthetic
CRSRPVESSCS

SEQ ID NO: 29 - protein, 12 aa, Synthetic
SCRSRPVESSCS

SEQ ID NO: 30 - protein, 11 aa, Synthetic
SCRARPVESSC

SEQ ID NO: 31 - protein, 11 aa, Synthetic
SCRSRPAESSC

SEQ ID NO: 32 - protein, 21 aa, Synthetic
IDPSSEAPGHSCRSRPVESSC

SEQ ID NO: 33 - protein, 25 aa, Synthetic
CRSRPVESSCSSKFSWDEYEQYKKE

SEQ ID NO: 34 - protein, 11 aa, Synthetic
SCRSRPVEASC

SEQ ID NO: 35 - protein, 11 aa, Synthetic
SCRSRPVESAC